European Patent Specification EP 4 023 772 B1, published February 28, 2024. Title: Composition for Detecting Mutations of 2019 Novel Coronavirus, Use and Kit Thereof. Applicant: Sansure Biotech Inc. Application EP20932880.6. The sequence listing filed with the application follows.

SEQUENCE LISTING (30 sequences)

SEQ ID NO: 1 - DNA, 24 bp, Artificial Sequence
  Artificial Sequence
gctgattttgacacatggttcatc

SEQ ID NO: 2 - DNA, 26 bp, Artificial Sequence
  Artificial Sequence
atcggtaattatacagtttccagatt

SEQ ID NO: 3 - DNA, 24 bp, Artificial Sequence
  Artificial Sequence
gctgattttgacacatggtatcgt

SEQ ID NO: 4 - DNA, 26 bp, Artificial Sequence
  Artificial Sequence
atcggtaattatacagtttcctttgc

SEQ ID NO: 5 - DNA, 23 bp, Artificial Sequence
  Artificial Sequence
ccattagttgtgcgtaatatcgt

SEQ ID NO: 6 - DNA, 27 bp, Artificial Sequence
  Artificial Sequence
cttgcccattgattgctgcagtcataa

SEQ ID NO: 7 - DNA, 24 bp, Artificial Sequence
  Artificial Sequence
caacacgaacgtcatgatactcta

SEQ ID NO: 8 - DNA, 26 bp, Artificial Sequence
  Artificial Sequence
attgccaggaacctaaattgggtagt

SEQ ID NO: 9 - DNA, 800 bp, Artificial Sequence
  Artificial Sequence
ttaattaaagttacacttgtgttcctttttgttgctgctattttctatttaataacacctgttcatgtcatgtctaaacatactgacttttcaagtgaaatcataggatacaaggctattgatggtggtgtcactcgtgacatagcatctacagatacttgttttgctaacaaacatgctgattttgacacatggtttagccagcgtggtggtagttatactaatgacaaagcttgcccattgattgctgcagtcataacaagagaagtgggttttgtcgtgcctggtttgcctggcacgatattacgcacaactaatggtgactttttgcatttcttacctagagtttttagtgcagttggtaacatctgttacacaccatcaaaacttatagagtacaccaagaatgtagtttacagtcatgtactcaacatcaaccatatgtagttgatgacccgtgtcctattcacttctattctaaatggtatattagagtaggagctagaaaatcagcacctttaattgaattgtgcgtggatgaggctggttctaaatcacccattcagtacatcgatatcggtaattatacagtttcctgtttaccttttacaattaattgccaggaacctaaattgggtagtcttgtagtgcgttgttcgttctatgaagactttttagagtatcatgacgttcgtgttgttttagatttcatctaaacgaacaaactaaaatgtctgataatggaccccaaaatcagcgaaatgcaccccgcattacgtttggtggaccctcagattcaa

SEQ ID NO: 10 - DNA, 800 bp, Artificial Sequence
  Artificial Sequence
ttaattaaagttacacttgtgttcctttttgttgctgctattttctatttaataacacctgttcatgtcatgtctaaacatactgacttttcaagtgaaatcataggatacaaggctattgatggtggtgtcactcgtgacatagcatctacagatacttgttttgctaacaaacatgctgattttgacacatggtttagtcagcgtggtggtagttatactaatgacaaagcttgcccattgattgctgcagtcataacaagagaagtgggttttgtcgtgcctggtttgcctggcacgatattacgcacaactaatggtgactttttgcatttcttacctagagtttttagtgcagttggtaacatctgttacacaccatcaaaacttatagagtacaccaagaatgtagtttacagtcatgtactcaacatcaaccatatgtagttgatgacccgtgtcctattcacttctattctaaatggtatattagagtaggagctagaaaatcagcacctttaattgaattgtgcgtggatgaggctggttctaaatcacccattcagtacatcgatatcggtaattatacagtttcctgttcaccttttacaattaattgccaggaacctaaattgggtagtcttgtagtgcgttgttcgttctatgaagactttttagagtatcatgacgttcgtgttgttttagatttcatctaaacgaacaaactaaaatgtctgataatggaccccaaaatcagcgaaatgcaccccgcattacgtttggtggaccctcagattcaa

SEQ ID NO: 11 - DNA, 24 bp, Artificial Sequence
  Artificial Sequence
gctgattttgacacatggtttagc

SEQ ID NO: 12 - DNA, 24 bp, Artificial Sequence
  Artificial Sequence
gctgattttgacacatggtttatc

SEQ ID NO: 13 - DNA, 24 bp, Artificial Sequence
  Artificial Sequence
gctgattttgacacatggtttcgc

SEQ ID NO: 14 - DNA, 24 bp, Artificial Sequence
  Artificial Sequence
gctgattttgacacatggtttctc

SEQ ID NO: 15 - DNA, 24 bp, Artificial Sequence
  Artificial Sequence
gctgattttgacacatggtctcgt

SEQ ID NO: 16 - DNA, 24 bp, Artificial Sequence
  Artificial Sequence
gctgattttgacacatggtttagt

SEQ ID NO: 17 - DNA, 24 bp, Artificial Sequence
  Artificial Sequence
gctgattttgacacatggtttcgt

SEQ ID NO: 18 - DNA, 24 bp, Artificial Sequence
  Artificial Sequence
gctgattttgacacatggtttatt

SEQ ID NO: 19 - DNA, 24 bp, Artificial Sequence
  Artificial Sequence
gctgattttgacacatggtttcat

SEQ ID NO: 20 - DNA, 24 bp, Artificial Sequence
  Artificial Sequence
gctgattttgacacatggttgatt

SEQ ID NO: 21 - DNA, 26 bp, Artificial Sequence
  Artificial Sequence
atcggtaattatacagtttcctgttt

SEQ ID NO: 22 - DNA, 26 bp, Artificial Sequence
  Artificial Sequence
atcggtaattatacagtttcctcttt

SEQ ID NO: 23 - DNA, 26 bp, Artificial Sequence
  Artificial Sequence
atcggtaattatacagtttcctggtt

SEQ ID NO: 24 - DNA, 26 bp, Artificial Sequence
  Artificial Sequence
atcggtaattatacagtttcctgggt

SEQ ID NO: 25 - DNA, 26 bp, Artificial Sequence
  Artificial Sequence
atcggtaattatacagtttcctctct

SEQ ID NO: 26 - DNA, 26 bp, Artificial Sequence
  Artificial Sequence
atcggtaattatacagtttcctgttc

SEQ ID NO: 27 - DNA, 26 bp, Artificial Sequence
  Artificial Sequence
atcggtaattatacagtttcctcttc

SEQ ID NO: 28 - DNA, 26 bp, Artificial Sequence
  Artificial Sequence
atcggtaattatacagtttcctggtc

SEQ ID NO: 29 - DNA, 26 bp, Artificial Sequence
  Artificial Sequence
atcggtaattatacagtttcctgagc

SEQ ID NO: 30 - DNA, 26 bp, Artificial Sequence
  Artificial Sequence
atcggtaattatacagtttccaggtc